European Patent Specification EP 3 591 039 B1, published July 8, 2026. Title: A method for separation of dopaminergic neural cells and a pharmaceutical composition comprising dopaminergic neural cells for the treatment of Parkinson's disease. Applicant: S-Biomedics. The sequence listing filed with the application follows.

SEQUENCE LISTING (53 sequences)

SEQ ID NO: 1 - DNA, 20 bp, Artificial Sequence
  GAPDH-F
caatgaccccttcattgacc

SEQ ID NO: 2 - DNA, 20 bp, Artificial Sequence
  GAPDH-R
ttgattttggagggatctcg

SEQ ID NO: 3 - DNA, 20 bp, Artificial Sequence
  OCT4-F
cctcacttcactgcactgta

SEQ ID NO: 4 - DNA, 20 bp, Artificial Sequence
  OCT4-R
caggttttctttccctagct

SEQ ID NO: 5 - DNA, 24 bp, Artificial Sequence
  SOX2-F
ttcacatgtcccagcactaccaga

SEQ ID NO: 6 - DNA, 26 bp, Artificial Sequence
  SOX2-R
tcacatgtgtgagaggggcagtgtgc

SEQ ID NO: 7 - DNA, 20 bp, Artificial Sequence
  NANOG-F
tgaacctcagctacaaacag

SEQ ID NO: 8 - DNA, 20 bp, Artificial Sequence
  NANOG-R
tggtggtaggaagagtaaag

SEQ ID NO: 9 - DNA, 24 bp, Artificial Sequence
  TET1-F
ctgcagctgtcttgatcgagttat

SEQ ID NO: 10 - DNA, 24 bp, Artificial Sequence
  TET1-R
ccttctttaccggtgtacactact

SEQ ID NO: 11 - DNA, 21 bp, Artificial Sequence
  REX1-F
tcacagtccagcaggtgtttg

SEQ ID NO: 12 - DNA, 20 bp, Artificial Sequence
  REX1-R
tcttgtctttgcccgtttct

SEQ ID NO: 13 - DNA, 20 bp, Artificial Sequence
  EN1-F
cgtggcttactccccattta

SEQ ID NO: 14 - DNA, 20 bp, Artificial Sequence
  EN1-R
tctcgctgtctctccctctc

SEQ ID NO: 15 - DNA, 20 bp, Artificial Sequence
  FOXA2-F
ccgttctccatcaacaacct

SEQ ID NO: 16 - DNA, 20 bp, Artificial Sequence
  FOXA2-R
ggggtagtgcatcacctgtt

SEQ ID NO: 17 - DNA, 20 bp, Artificial Sequence
  LMX1A-F
cgcatcgtttcttctcctct

SEQ ID NO: 18 - DNA, 20 bp, Artificial Sequence
  LMX1A-R
cagacagacttggggctcac

SEQ ID NO: 19 - DNA, 31 bp, Artificial Sequence
  eGFP-F
catcaaggtgaacttcaagatccgccacaac

SEQ ID NO: 20 - DNA, 31 bp, Artificial Sequence
  eGFP-R
cttgtacagctcgtccatgccgagagtgatc

SEQ ID NO: 21 - DNA, 17 bp, Artificial Sequence
  PITX3-F
gccaaccttagtccgtg

SEQ ID NO: 22 - DNA, 17 bp, Artificial Sequence
  PITX3-R
gcaagccagtcaaaatg

SEQ ID NO: 23 - DNA, 20 bp, Artificial Sequence
  mCherry-F
actacgacgctgaggtcaag

SEQ ID NO: 24 - DNA, 20 bp, Artificial Sequence
  mCherry-R
gtgtagtcctcgttgtggga

SEQ ID NO: 25 - DNA, 22 bp, Artificial Sequence
  OTX2-F
ggaagcactgtttgccaagacc

SEQ ID NO: 26 - DNA, 22 bp, Artificial Sequence
  OTX2-R
ctgttgttggcggcacttagct

SEQ ID NO: 27 - DNA, 20 bp, Artificial Sequence
  FOXA1-F
gggcagggtggctccaggat

SEQ ID NO: 28 - DNA, 20 bp, Artificial Sequence
  FOXA1-R
tgctgaccgggacggaggag

SEQ ID NO: 29 - DNA, 20 bp, Artificial Sequence
  SIM1-F
aaagggggccaaatcccggc

SEQ ID NO: 30 - DNA, 20 bp, Artificial Sequence
  SIM1-R
tccgccccactggctgtcat

SEQ ID NO: 31 - DNA, 20 bp, Artificial Sequence
  LHX1-F
aggtgaaacactttgctccg

SEQ ID NO: 32 - DNA, 20 bp, Artificial Sequence
  LHX1-R
ctccagggaaggcaaactct

SEQ ID NO: 33 - DNA, 20 bp, Artificial Sequence
  LMX1B-F
aggtgaaacactttgctccg

SEQ ID NO: 34 - DNA, 20 bp, Artificial Sequence
  LMX1B-R
tcaggaggcgaagtaggaac

SEQ ID NO: 35 - DNA, 22 bp, Artificial Sequence
  NKX2.2-F
ccttctacgacagcagcgacaa

SEQ ID NO: 36 - DNA, 22 bp, Artificial Sequence
  NKX2.2-R
acttggagcttgagtcctgagg

SEQ ID NO: 37 - DNA, 20 bp, Artificial Sequence
  NKX6.1-F
cgagtcctgcttcttcttgg

SEQ ID NO: 38 - DNA, 20 bp, Artificial Sequence
  NKX6.1-R
ggggatgacagagagtcagg

SEQ ID NO: 39 - DNA, 22 bp, Artificial Sequence
  NURR1-F
aaactgcccagtggacaagcgt

SEQ ID NO: 40 - DNA, 22 bp, Artificial Sequence
  NURR1-R
gctcttcggtttcgagggcaaa

SEQ ID NO: 41 - DNA, 22 bp, Artificial Sequence
  TH-F
gctggacaagtgtcatcacctg

SEQ ID NO: 42 - DNA, 22 bp, Artificial Sequence
  TH-R
cctgtactggaaggcgatctca

SEQ ID NO: 43 - DNA, 22 bp, Artificial Sequence
  DAT-F
cctcaacgacacttttgggacc

SEQ ID NO: 44 - DNA, 22 bp, Artificial Sequence
  DAT-R
agtagagcagcacgatgaccag

SEQ ID NO: 45 - DNA, 22 bp, Artificial Sequence
  VMAT2-F
gctatgccttcctgctgattgc

SEQ ID NO: 46 - DNA, 22 bp, Artificial Sequence
  VMAT2-R
ccaaggcgattcccatgacgtt

SEQ ID NO: 47 - DNA, 23 bp, Artificial Sequence
  HTR2B-F
gctggttggattgtttgtgatgc

SEQ ID NO: 48 - DNA, 23 bp, Artificial Sequence
  HTR2B-R
ccactgaaatggcacagagatgc

SEQ ID NO: 49 - DNA, 22 bp, Artificial Sequence
  NeuN-F
tacgcagcctacagatacgctc

SEQ ID NO: 50 - DNA, 22 bp, Artificial Sequence
  NeuN-R
tggttccaatgctgtaggtcgc

SEQ ID NO: 51 - DNA, 22 bp, Artificial Sequence
  MAP2-F
aggctgtagcagtcctgaaagg

SEQ ID NO: 52 - DNA, 22 bp, Artificial Sequence
  MAP2-R
cttcctccactgtgacagtctg

SEQ ID NO: 53 - DNA, 8823 bp, Trophoblast glycoprotein
actaaaggcacatgtcccaggcacaagcctcaggatccttatttgatcttttttaatacgaccaggtcttaaatttccgaaccatgttttccctaattgccattttctctctaaaatgaagaagcctggaagaaccttcttatcccttcggggaaattatttaattgggacaaaggggatgtggagttacagagagcaacgatagggctttcagaacccaaaacctgtctggtataataacagatccttccggtaaccaaccattcaatttgtccctctccccaaccccatcctctccatcaccatctgccagatgccccctgggacaatcgactttgaaaccaaacttctctcccaggtcagctcctgcaatccccactcctcatccttggagctttctccacagaagtgacttgacacaccgcgctacatctggggaggggggcgggtccgctttccgggagactcaagtctttgctatttgccttttgtttctgggatgcctttggctgcctttctcttccatctgcttttaattttggtaagagaaaagctaatgaatcaggaatgaatctcctctccactaatcttttttttttctttctctctctctctctcttaaagttggcgcgctctcttcacaagttccatcactacccaagaagtgagggggcgggggggacaggcgggaaggcattaattacacctaaatctgaagtttgcggcctcaagtaccactttgatggggagagcttctgaagcttccatacaacctgccgtgcctttgctgctgccgcagtagattttcagctcatttctttctgctgctgcttcgcgctgctctgtcatgcctaaatctatctcgtcactgccaaaggtgcctgaatcagggtgaattccacgagattcaccagcggttttgctccagtccaaggtaaatacagtatgcaaaatgaggaaccacccaaggatgtcggggaggggggagagaaagggattccctcaccttttccggcacattcctcgttaatttccaccaggaggaggcgcgcagcccagctcccctagtctctcttcttaaatccccctacctacggctgccgaggttggccgcgcgtcgggaatctccccgacagtcctggccctcccccgccccccgggttggtttttcccagctgcggaggttgggaggttgggccaggggctggggtgcgaagagagtcggcgcccgcaacgcggagccgggaagtcgtcgctactctggtggaactcagagttggttctggaggcggcggacgcggaggtgagcagtgggagcccgcggcctgggagagacccgggaggcgtcgttggggcccctccccatcctcgggtggagagtagggttggttcgggttgccactgtaccccgagtcccactgctgctttgttcccagactctcccctcctctttggagatgacttgaacccctttgagatccgaggggctggcggggcgcgggctggggggcgacagttgtagctccacttcctgctaatgcgagaaggtacaaaaagagatcaaaaagtcctgtaacctgaaacttccctcgcatcctaaccgggacctggtggagaggtctgggcgggggcggagacacccggaggccgaccttccgccgaggcggtgcaggaaggaacgggagagggagaagtttggtagggaaggaattggggattaagcggtaagttagacgcgggagacgagtctcctcgggaaaggcggagggcgggaggccggtcgggtttatttagtgtgggccagggaagaaggaagactttgcggtctgggtgtcggatgcgcgtccccctccggagtaaaagtgaccggaggggttggggaggcgaggccggggcgggcttttggaaggaggtctctgggacagactggagacgactagactcgaaaaggccggtttttgcactccggaagccgcggcagccaccgctgttcacgcctctctcctgcttgtcccaggtccctcagaggatccagcgaggggcgccaacaagaggcgaagaggtggcaccagggcggcggcaggaagaggagcgggagcaggagcgcggagcggagcgtcccgacccgccgtgcgtactttctggagggaaggggcgggggaatcggcccctgagggaagcgcccggtggcgagggggttagccaagttccggctgcggcgccactccctcggttccacgagaggaaagttttttttttccagacgcttccgccggctcgcgccctccgggcccagcctcccgagccttcggagcgggcgccgtcccagcccagctccggggaaacgcgagccgcgatgcctggggggtgctcccggggccccgccgccggggacgggcgtctgcggctggcgcgactagcgctggtactcctgggctgggtctcctcgtcttctcccacctcctcggcatcctccttctcctcctcggcgccgttcctggcttccgccgtgtccgcccagcccccgctgccggaccagtgccccgcgctgtgcgagtgctccgaggcagcgcgcacagtcaagtgcgttaaccgcaatctgaccgaggtgcccacggacctgcccgcctacgtgcgcaacctcttccttaccggcaaccagctggccgtgctccctgccggcgccttcgcccgccggccgccgctggcggagctggccgcgctcaacctcagcggcagccgcctggacgaggtgcgcgcgggcgccttcgagcatctgcccagcctgcgccagctcgacctcagccacaacccactggccgacctcagtcccttcgctttctcgggcagcaatgccagcgtctcggcccccagtccccttgtggaactgatcctgaaccacatcgtgccccctgaagatgagcggcagaaccggagcttcgagggcatggtggtggcggccctgctggcgggccgtgcactgcaggggctccgccgcttggagctggccagcaaccacttcctttacctgccgcgggatgtgctggcccaactgcccagcctcaggcacctggacttaagtaataattcgctggtgagcctgacctacgtgtccttccgcaacctgacacatctagaaagcctccacctggaggacaatgccctcaaggtccttcacaatggcaccctggctgagttgcaaggtctaccccacattagggttttcctggacaacaatccctgggtctgcgactgccacatggcagacatggtgacctggctcaaggaaacagaggtagtgcagggcaaagaccggctcacctgtgcatatccggaaaaaatgaggaatcgggtcctcttggaactcaacagtgctgacctggactgtgacccgattcttcccccatccctgcaaacctcttatgtcttcctgggtattgttttagccctgataggcgctattttcctcctggttttgtatttgaaccgcaaggggataaaaaagtggatgcataacatcagagatgcctgcagggatcacatggaagggtatcattacagatatgaaatcaatgcggaccccagattaacgaacctcagttctaactcggatgtctgagaaatattagaggacagaccaaggacaactctgcatgagatgtagacttaagctttatccctactaggcttgctccactttcatcctccactatagatacaacggactttgactaaaagcagtgaaggggatttgcttccttgttatgtaaagtttctcggtgtgttctgttaatgtaagacgatgaacagttgtgtatagtgttttaccctcttctttttcttggaactcctcaacacgtatggagggatttttcaggtttcagcatgaacatgggcttcttgctgtctgtctctctctcagtacagttcaaggtgtagcaagtgtacccacacagatagcattcaacaaaagctgcctcaactttttcgagaaaaatactttattcataaatatcagttttattctcatgtacctaagttgtggagaaaataattgcatcctataaactgcctgcagacgttagcaggctcttcaaaataactccatggtgcacaggagcacctgcatccaagagcatgcttacattttactgttctgcatattacaaaaaataacttgcaacttcataacttctttgacaaagtaaattacttttttgattgcagtttatatgaaaatgtactgatttttttttaataaactgcatcgagatccaaccgactgaattgttaaaaaaaaaaaaaataaagattcttaaaagaattacagtgtgtgcaagtttgctttgaaaaaaggatgaagggcaggagtattcaatggtcttggttccgatgataattattacttaacatagctgagaatcaaactgtagcaatgtctaatataaatagacttgggagatcgttttgaaatggtggatccttttagtatttaaatggagagtttgagtattcatgtgactgtatggtcccaaagttaatgctatttatgaaacagttttgtaagaacataatgaagttggtaaaagctaagcgttctgcacaataaacagttcccagtttggggctttttcaaggctaatgaagttattgttggtctagaaaaatagtatttacttaataaaactctgtttgaaattgttctgtggatttttagagcagaatttgaaacaaatgtaatgcaaataaatataaagataaagtgtcttaaagacaatattctgaaataaaagatataaaatataatttaaaaaatatttctcaatgtcttaatgtaaattgaaacttagattttcttgaggatattttcaaaaaaacatttaaagtggaacataaatgttctttagtttatcagagacccagctaatatgtttaaaaagttgacttgacatggttgaatatgaacttgaggaaataaccacagataaatgtctacatctgtaaacacgtgtctcaagtatttataggttcttatcttcagttcagtgtttaagaatttgaggatattttgattttagctaagctgttcataatgtaagtatatacacctttgtgaagaataaatcacatttaggtgtaaatacaggcaatcattaattgatacatccataatatacaaggcttttattattttttcagtttattatctgtcatttaatctgaaaagtaaattccattaatcagtcttcaggctcttttatcaagtgatttaaatgtagccattattgcttaactgaaagtattaggtaaacttgcatcagtaagtcttagggcttgcttttcctttgaactggttatgtccttcagtgctttatgtttgaaataaaatctacattttcatatttttataaataaaataggatcagatagtattttaggttctagaaatctttgctgattccttctttgaattaaattcagaaattttcaaagtagggctaaaaataagtaaatcttcctttttataggttagaatatatagtcagaatacaaagctgtaattccttaaattccatcaggcttgttttgtgaaatatagtatttattatttaagggttatatttcagatcctataattacctcagaaaaagctaaatatttggcacttaaaattccatcaaacagtttaagtgttcatcagaaattcctaaactgtctggttgccattatttggtaagaacaatgagatactaatctgtcaaaaatagtgaccactatcttagtaaactgttgatggacttagtaagtcttctgatattgtaggaaacaaattataatattgatagagcctctattgagaagaattgtttcttcatcacatgataatctaacagtttaaagtggagctttatctaagaaccagggaagcagtagattcattagtctagcttttctcatcaactctttgaagcaatgatgaatctgataaagtgaagccaagttttccctgttaggtagatggcttctttgaagttataatttattgcttctttttcatccccctacttattctcttgtttggactttccaattgctactgctttgttttccatcacatcactccttcctgttctccaaaatatggaaataaaaaagtcaattaaaagaacaccttattcttaagataaaaaattgttattatttgacaactaattaatgttttgcagccctaatattcttaagtctataagcttataaaacattctaagttccttggaagatagaggctatataaattcaataagtataagggaatatgggaaaaataaaagtatcactttatttaaaaataagacaagtctgtttgttttaaatactgttcttactattaatgcattgttgactctagaaacctgcaagtatccatttttaaaattttattttagttggtaatactctttattactgaacgtaaaattttcaacataaaacacccttcatttatcctttacaagtttcatttgaagaaagttagaaaaaatacttagaaattcaaggacttgatatatcccttaatttagaaagctattcaactatcccataaatttctatttaaagtagcaaaaattttaggataatacagctatttggccctgaattataactgccccctttgattgtaaccattcagtttgcagcattcgtttttgtaatagcagtttggctgctatgggtgtgattcaatggtaacctacaaggcaaatttgtacaggagctgacagatttttctaacaaaataaggagactttgaagcacattgaataggagtttttaaatgaataggattttttaaaggaaaaagagtaggagcttgggggggaaggctggttgaaataaatgagcaaatcacaaataataaatcctttagaaataccttgattggcagtaagtgtggattatgctcatctcagtatttaattagaaataacttacctttgtcttttgtctttttaattaaagtggctgtaaaaaagaaggtccagatgaactgagattgtttgcttaggaattctgttttactcttttccttttacctgatgttctaaaacagggcttaccttgttgaggaccttagaggctttgcaattctagattgtgattctttcatatcattttagtttttctcccaagactacactaaaggagacatcacgagatttgcaaggttaaaaacaattctgcacgtgcttcctcctgctcccaaatccggtcatccacctttcagagcagcaccgtaaagtgaagacagacatttattagatgaaattctggtttcacttttacacttgtgcaagcatttttaacagtaaaggagaggaaagggaggaatttatatttctagataatatatgaaaattaccttgatattgtatttttaagatctttcaccaatactgcagtgctgcactagaaataattagtttaagaaaatacattcaacattgtccaggtgatcctgtcaccttttagatgacgaaaaacatcttgaggatgttttgtacagttattttcccattgttactcttagagacttttgtttcaaaaaggcaggctcattttattttgttttatcttagaacattttagcagctctttgtcatgggttaaaaaaatctagaattaaaaaaatgtttaatatatgatttatataattttgacaagaatacaaattcttagtcgttcaaaattggaagcgctcttagaagtgtcaagctcagctttccattccacaaatgaagtaactggtaactgtgacttattatgttatacagtgacagttattatgttatacagtgtcagttatacagtgacaaccaggacaaaatcctagggttctagattccccttctggtgctctttttaccagatgatggcattactaattgcctaccttgaggcctttgaaatcaccatgtctgataaaaacatgcaattgctttggtgaatttgtttgttttattgttgttgctttgagtgaatgcttcagtttgctctagattttactttgttaaaaattaccatgttttaacccccgaaaacatttaatgtttttgaaatgattttttcataacaatcttatgagtctattatataataggaagtattttggaaatttaatggtgatatttctttggaaaagaaaaataaaaactctggaatgcagtgctggtttgtataattcaaccttaaatgtgagttaagctcagctggtgagaaaactaaacaaatgagaccaagttcgtgaccattaagtcaatcagtcaccaggtgagacagtcagctttgcattctctgctgtgttctcctagctcacgcccactccaggtgcatgctgccatcctctaagggcctggaccaaacagggaagttagttaaatcaatgcaaatccattatcaccctggaaaaccaggggactgaccagccgaacactgccagcttggctgctgaagtgccagtttactgtctttacatatgcaggacacacactacatctcaattttctcacatcatatgtagtatttatgctgcagattgcaaaaggcttataatttatgtgaattttgggaagctagcatgagtacctttcagggtattgcatgggaaattaattaggtttactttattattttaaaaaagtgtgggttaagattaagcaacatgattactatatcatacacttacacgtaaatgtttataaaaacaaatacagtttatatttagctgacattttatgataggacttacttgtggttcacaattta